European Patent Specification EP 3 428 181 B1, published October 8, 2025. Title: ANTI-INFLAMMATORY PEPTIDES AND COMPOSITION COMPRISING THE SAME. Applicant: KAEL-GemVax Co., Ltd KIM, Sang Jae. The sequence listing filed with the application follows.

SEQUENCE LISTING (180 sequences)

SEQ ID NO: 1 - protein, 16 aa, Homo sapiens
EARPALLTSRLRFIPK

SEQ ID NO: 2 - protein, 17 aa, Homo sapiens
REARPALLTSRLRFIPK

SEQ ID NO: 3 - protein, 18 aa, Homo sapiens
HREARPALLTSRLRFIPK

SEQ ID NO: 4 - protein, 19 aa, Homo sapiens
QHREARPALLTSRLRFIPK

SEQ ID NO: 5 - protein, 20 aa, Homo sapiens
RQHREARPALLTSRLRFIPK

SEQ ID NO: 6 - protein, 21 aa, Homo sapiens
VRQHREARPALLTSRLRFIPK

SEQ ID NO: 7 - protein, 22 aa, Homo sapiens
EVRQHREARPALLTSRLRFIPK

SEQ ID NO: 8 - protein, 23 aa, Homo sapiens
AEVRQHREARPALLTSRLRFIPK

SEQ ID NO: 9 - protein, 24 aa, Homo sapiens
EAEVRQHREARPALLTSRLRFIPK

SEQ ID NO: 10 - protein, 25 aa, Homo sapiens
SEAEVRQHREARPALLTSRLRFIPK

SEQ ID NO: 11 - protein, 26 aa, Homo sapiens
LSEAEVRQHREARPALLTSRLRFIPK

SEQ ID NO: 12 - protein, 27 aa, Homo sapiens
ELSEAEVRQHREARPALLTSRLRFIPK

SEQ ID NO: 13 - protein, 28 aa, Homo sapiens
RELSEAEVRQHREARPALLTSRLRFIPK

SEQ ID NO: 14 - protein, 29 aa, Homo sapiens
LRELSEAEVRQHREARPALLTSRLRFIPK

SEQ ID NO: 15 - protein, 30 aa, Homo sapiens
QLRELSEAEVRQHREARPALLTSRLRFIPK

SEQ ID NO: 16 - protein, 18 aa, Homo sapiens
REARPALLTSRLRFIPKP

SEQ ID NO: 17 - protein, 19 aa, Homo sapiens
HREARPALLTSRLRFIPKP

SEQ ID NO: 18 - protein, 20 aa, Homo sapiens
HREARPALLTSRLRFIPKPD

SEQ ID NO: 19 - protein, 19 aa, Homo sapiens
REARPALLTSRLRFIPKPD

SEQ ID NO: 20 - protein, 20 aa, Homo sapiens
QHREARPALLTSRLRFIPKP

SEQ ID NO: 21 - protein, 21 aa, Homo sapiens
QHREARPALLTSRLRFIPKPD

SEQ ID NO: 22 - protein, 22 aa, Homo sapiens
QHREARPALLTSRLRFIPKPDG

SEQ ID NO: 23 - protein, 21 aa, Homo sapiens
HREARPALLTSRLRFIPKPDG

SEQ ID NO: 24 - protein, 20 aa, Homo sapiens
REARPALLTSRLRFIPKPDG

SEQ ID NO: 25 - protein, 21 aa, Homo sapiens
RQHREARPALLTSRLRFIPKP

SEQ ID NO: 26 - protein, 22 aa, Homo sapiens
RQHREARPALLTSRLRFIPKPD

SEQ ID NO: 27 - protein, 23 aa, Homo sapiens
RQHREARPALLTSRLRFIPKPDG

SEQ ID NO: 28 - protein, 24 aa, Homo sapiens
RQHREARPALLTSRLRFIPKPDGL

SEQ ID NO: 29 - protein, 23 aa, Homo sapiens
QHREARPALLTSRLRFIPKPDGL

SEQ ID NO: 30 - protein, 22 aa, Homo sapiens
HREARPALLTSRLRFIPKPDGL

SEQ ID NO: 31 - protein, 21 aa, Homo sapiens
REARPALLTSRLRFIPKPDGL

SEQ ID NO: 32 - protein, 22 aa, Homo sapiens
VRQHREARPALLTSRLRFIPKP

SEQ ID NO: 33 - protein, 23 aa, Homo sapiens
VRQHREARPALLTSRLRFIPKPD

SEQ ID NO: 34 - protein, 24 aa, Homo sapiens
VRQHREARPALLTSRLRFIPKPDG

SEQ ID NO: 35 - protein, 25 aa, Homo sapiens
VRQHREARPALLTSRLRFIPKPDGL

SEQ ID NO: 36 - protein, 26 aa, Homo sapiens
VRQHREARPALLTSRLRFIPKPDGLR

SEQ ID NO: 37 - protein, 25 aa, Homo sapiens
RQHREARPALLTSRLRFIPKPDGLR

SEQ ID NO: 38 - protein, 24 aa, Homo sapiens
QHREARPALLTSRLRFIPKPDGLR

SEQ ID NO: 39 - protein, 23 aa, Homo sapiens
HREARPALLTSRLRFIPKPDGLR

SEQ ID NO: 40 - protein, 22 aa, Homo sapiens
REARPALLTSRLRFIPKPDGLR

SEQ ID NO: 41 - protein, 23 aa, Homo sapiens
EVRQHREARPALLTSRLRFIPKP

SEQ ID NO: 42 - protein, 24 aa, Homo sapiens
EVRQHREARPALLTSRLRFIPKPD

SEQ ID NO: 43 - protein, 25 aa, Homo sapiens
EVRQHREARPALLTSRLRFIPKPDG

SEQ ID NO: 44 - protein, 26 aa, Homo sapiens
EVRQHREARPALLTSRLRFIPKPDGL

SEQ ID NO: 45 - protein, 27 aa, Homo sapiens
EVRQHREARPALLTSRLRFIPKPDGLR

SEQ ID NO: 46 - protein, 28 aa, Homo sapiens
EVRQHREARPALLTSRLRFIPKPDGLRP

SEQ ID NO: 47 - protein, 27 aa, Homo sapiens
VRQHREARPALLTSRLRFIPKPDGLRP

SEQ ID NO: 48 - protein, 26 aa, Homo sapiens
RQHREARPALLTSRLRFIPKPDGLRP

SEQ ID NO: 49 - protein, 25 aa, Homo sapiens
QHREARPALLTSRLRFIPKPDGLRP

SEQ ID NO: 50 - protein, 24 aa, Homo sapiens
HREARPALLTSRLRFIPKPDGLRP

SEQ ID NO: 51 - protein, 23 aa, Homo sapiens
REARPALLTSRLRFIPKPDGLRP

SEQ ID NO: 52 - protein, 24 aa, Homo sapiens
AEVRQHREARPALLTSRLRFIPKP

SEQ ID NO: 53 - protein, 25 aa, Homo sapiens
AEVRQHREARPALLTSRLRFIPKPD

SEQ ID NO: 54 - protein, 26 aa, Homo sapiens
AEVRQHREARPALLTSRLRFIPKPDG

SEQ ID NO: 55 - protein, 27 aa, Homo sapiens
AEVRQHREARPALLTSRLRFIPKPDGL

SEQ ID NO: 56 - protein, 28 aa, Homo sapiens
AEVRQHREARPALLTSRLRFIPKPDGLR

SEQ ID NO: 57 - protein, 29 aa, Homo sapiens
AEVRQHREARPALLTSRLRFIPKPDGLRP

SEQ ID NO: 58 - protein, 30 aa, Homo sapiens
AEVRQHREARPALLTSRLRFIPKPDGLRPI

SEQ ID NO: 59 - protein, 29 aa, Homo sapiens
EVRQHREARPALLTSRLRFIPKPDGLRPI

SEQ ID NO: 60 - protein, 28 aa, Homo sapiens
VRQHREARPALLTSRLRFIPKPDGLRPI

SEQ ID NO: 61 - protein, 27 aa, Homo sapiens
RQHREARPALLTSRLRFIPKPDGLRPI

SEQ ID NO: 62 - protein, 26 aa, Homo sapiens
QHREARPALLTSRLRFIPKPDGLRPI

SEQ ID NO: 63 - protein, 25 aa, Homo sapiens
HREARPALLTSRLRFIPKPDGLRPI

SEQ ID NO: 64 - protein, 24 aa, Homo sapiens
REARPALLTSRLRFIPKPDGLRPI

SEQ ID NO: 65 - protein, 17 aa, Homo sapiens
EARPALLTSRLRFIPKP

SEQ ID NO: 66 - protein, 18 aa, Homo sapiens
EARPALLTSRLRFIPKPD

SEQ ID NO: 67 - protein, 19 aa, Homo sapiens
EARPALLTSRLRFIPKPDG

SEQ ID NO: 68 - protein, 21 aa, Homo sapiens
EARPALLTSRLRFIPKPDGLR

SEQ ID NO: 69 - protein, 22 aa, Homo sapiens
EARPALLTSRLRFIPKPDGLRP

SEQ ID NO: 70 - protein, 23 aa, Homo sapiens
EARPALLTSRLRFIPKPDGLRPI

SEQ ID NO: 71 - protein, 24 aa, Homo sapiens
EARPALLTSRLRFIPKPDGLRPIV

SEQ ID NO: 72 - protein, 25 aa, Homo sapiens
EARPALLTSRLRFIPKPDGLRPIVN

SEQ ID NO: 73 - protein, 26 aa, Homo sapiens
EARPALLTSRLRFIPKPDGLRPIVNM

SEQ ID NO: 74 - protein, 27 aa, Homo sapiens
EARPALLTSRLRFIPKPDGLRPIVNMD

SEQ ID NO: 75 - protein, 28 aa, Homo sapiens
EARPALLTSRLRFIPKPDGLRPIVNMDY

SEQ ID NO: 76 - protein, 29 aa, Homo sapiens
EARPALLTSRLRFIPKPDGLRPIVNMDYV

SEQ ID NO: 77 - protein, 30 aa, Homo sapiens
EARPALLTSRLRFIPKPDGLRPIVNMDYVV

SEQ ID NO: 78 - protein, 15 aa, Homo sapiens
EARPALLTSRLRFIP

SEQ ID NO: 79 - protein, 14 aa, Homo sapiens
EARPALLTSRLRFI

SEQ ID NO: 80 - protein, 13 aa, Homo sapiens
EARPALLTSRLRF

SEQ ID NO: 81 - protein, 12 aa, Homo sapiens
EARPALLTSRLR

SEQ ID NO: 82 - protein, 11 aa, Homo sapiens
EARPALLTSRL

SEQ ID NO: 83 - protein, 10 aa, Homo sapiens
EARPALLTSR

SEQ ID NO: 84 - protein, 9 aa, Homo sapiens
EARPALLTS

SEQ ID NO: 85 - protein, 8 aa, Homo sapiens
EARPALLT

SEQ ID NO: 86 - protein, 7 aa, Homo sapiens
EARPALL

SEQ ID NO: 87 - protein, 6 aa, Homo sapiens
EARPAL

SEQ ID NO: 88 - protein, 5 aa, Homo sapiens
EARPA

SEQ ID NO: 89 - protein, 4 aa, Homo sapiens
EARP

SEQ ID NO: 90 - protein, 3 aa, Homo sapiens
EAR

SEQ ID NO: 91 - protein, 15 aa, Homo sapiens
ARPALLTSRLRFIPK

SEQ ID NO: 92 - protein, 14 aa, Homo sapiens
RPALLTSRLRFIPK

SEQ ID NO: 93 - protein, 13 aa, Homo sapiens
PALLTSRLRFIPK

SEQ ID NO: 94 - protein, 12 aa, Homo sapiens
ALLTSRLRFIPK

SEQ ID NO: 95 - protein, 11 aa, Homo sapiens
LLTSRLRFIPK

SEQ ID NO: 96 - protein, 10 aa, Homo sapiens
LTSRLRFIPK

SEQ ID NO: 97 - protein, 9 aa, Homo sapiens
TSRLRFIPK

SEQ ID NO: 98 - protein, 8 aa, Homo sapiens
SRLRFIPK

SEQ ID NO: 99 - protein, 7 aa, Homo sapiens
RLRFIPK

SEQ ID NO: 100 - protein, 6 aa, Homo sapiens
LRFIPK

SEQ ID NO: 101 - protein, 5 aa, Homo sapiens
RFIPK

SEQ ID NO: 102 - protein, 4 aa, Homo sapiens
FIPK

SEQ ID NO: 103 - protein, 3 aa, Homo sapiens
IPK

SEQ ID NO: 104 - protein, 14 aa, Homo sapiens
ARPALLTSRLRFIP

SEQ ID NO: 105 - protein, 12 aa, Homo sapiens
RPALLTSRLRFI

SEQ ID NO: 106 - protein, 10 aa, Homo sapiens
PALLTSRLRF

SEQ ID NO: 107 - protein, 8 aa, Homo sapiens
ALLTSRLR

SEQ ID NO: 108 - protein, 6 aa, Homo sapiens
LLTSRL

SEQ ID NO: 109 - protein, 4 aa, Homo sapiens
LTSR

SEQ ID NO: 110 - protein, 13 aa, Homo sapiens
ARPALLTSRLRFI

SEQ ID NO: 111 - protein, 12 aa, Homo sapiens
ARPALLTSRLRF

SEQ ID NO: 112 - protein, 11 aa, Homo sapiens
ARPALLTSRLR

SEQ ID NO: 113 - protein, 10 aa, Homo sapiens
ARPALLTSRL

SEQ ID NO: 114 - protein, 9 aa, Homo sapiens
ARPALLTSR

SEQ ID NO: 115 - protein, 8 aa, Homo sapiens
ARPALLTS

SEQ ID NO: 116 - protein, 7 aa, Homo sapiens
ARPALLT

SEQ ID NO: 117 - protein, 6 aa, Homo sapiens
ARPALL

SEQ ID NO: 118 - protein, 5 aa, Homo sapiens
ARPAL

SEQ ID NO: 119 - protein, 4 aa, Homo sapiens
ARPA

SEQ ID NO: 120 - protein, 3 aa, Homo sapiens
ARP

SEQ ID NO: 121 - protein, 13 aa, Homo sapiens
RPALLTSRLRFIP

SEQ ID NO: 122 - protein, 11 aa, Homo sapiens
RPALLTSRLRF

SEQ ID NO: 123 - protein, 10 aa, Homo sapiens
RPALLTSRLR

SEQ ID NO: 124 - protein, 8 aa, Homo sapiens
RPALLTSR

SEQ ID NO: 125 - protein, 7 aa, Homo sapiens
RPALLTS

SEQ ID NO: 126 - protein, 6 aa, Homo sapiens
RPALLT

SEQ ID NO: 127 - protein, 5 aa, Homo sapiens
RPALL

SEQ ID NO: 128 - protein, 4 aa, Homo sapiens
RPAL

SEQ ID NO: 129 - protein, 3 aa, Homo sapiens
RPA

SEQ ID NO: 130 - protein, 12 aa, Homo sapiens
PALLTSRLRFIP

SEQ ID NO: 131 - protein, 11 aa, Homo sapiens
PALLTSRLRFI

SEQ ID NO: 132 - protein, 9 aa, Homo sapiens
PALLTSRLR

SEQ ID NO: 133 - protein, 8 aa, Homo sapiens
PALLTSRL

SEQ ID NO: 134 - protein, 7 aa, Homo sapiens
PALLTSR

SEQ ID NO: 135 - protein, 6 aa, Homo sapiens
PALLTS

SEQ ID NO: 136 - protein, 5 aa, Homo sapiens
PALLT

SEQ ID NO: 137 - protein, 4 aa, Homo sapiens
PALL

SEQ ID NO: 138 - protein, 3 aa, Homo sapiens
PAL

SEQ ID NO: 139 - protein, 11 aa, Homo sapiens
ALLTSRLRFIP

SEQ ID NO: 140 - protein, 9 aa, Homo sapiens
ALLTSRLRF

SEQ ID NO: 141 - protein, 7 aa, Homo sapiens
ALLTSRL

SEQ ID NO: 142 - protein, 6 aa, Homo sapiens
ALLTSR

SEQ ID NO: 143 - protein, 5 aa, Homo sapiens
ALLTS

SEQ ID NO: 144 - protein, 4 aa, Homo sapiens
ALLT

SEQ ID NO: 145 - protein, 3 aa, Homo sapiens
ALL

SEQ ID NO: 146 - protein, 10 aa, Homo sapiens
LLTSRLRFIP

SEQ ID NO: 147 - protein, 9 aa, Homo sapiens
LLTSRLRFI

SEQ ID NO: 148 - protein, 8 aa, Homo sapiens
LLTSRLRF

SEQ ID NO: 149 - protein, 7 aa, Homo sapiens
LLTSRLR

SEQ ID NO: 150 - protein, 5 aa, Homo sapiens
LLTSR

SEQ ID NO: 151 - protein, 4 aa, Homo sapiens
LLTS

SEQ ID NO: 152 - protein, 3 aa, Homo sapiens
LLT

SEQ ID NO: 153 - protein, 9 aa, Homo sapiens
LTSRLRFIP

SEQ ID NO: 154 - protein, 8 aa, Homo sapiens
LTSRLRFI

SEQ ID NO: 155 - protein, 7 aa, Homo sapiens
LTSRLRF

SEQ ID NO: 156 - protein, 6 aa, Homo sapiens
LTSRLR

SEQ ID NO: 157 - protein, 5 aa, Homo sapiens
LTSRL

SEQ ID NO: 158 - protein, 3 aa, Homo sapiens
LTS

SEQ ID NO: 159 - protein, 8 aa, Homo sapiens
TSRLRFIP

SEQ ID NO: 160 - protein, 7 aa, Homo sapiens
TSRLRFI

SEQ ID NO: 161 - protein, 6 aa, Homo sapiens
TSRLRF

SEQ ID NO: 162 - protein, 5 aa, Homo sapiens
TSRLR

SEQ ID NO: 163 - protein, 4 aa, Homo sapiens
TSRL

SEQ ID NO: 164 - protein, 3 aa, Homo sapiens
TSR

SEQ ID NO: 165 - protein, 7 aa, Homo sapiens
SRLRFIP

SEQ ID NO: 166 - protein, 6 aa, Homo sapiens
SRLRFI

SEQ ID NO: 167 - protein, 5 aa, Homo sapiens
SRLRF

SEQ ID NO: 168 - protein, 4 aa, Homo sapiens
SRLR

SEQ ID NO: 169 - protein, 3 aa, Homo sapiens
SRL

SEQ ID NO: 170 - protein, 6 aa, Homo sapiens
RLRFIP

SEQ ID NO: 171 - protein, 5 aa, Homo sapiens
RLRFI

SEQ ID NO: 172 - protein, 4 aa, Homo sapiens
RLRF

SEQ ID NO: 173 - protein, 3 aa, Homo sapiens
RLR

SEQ ID NO: 174 - protein, 5 aa, Homo sapiens
LRFIP

SEQ ID NO: 175 - protein, 4 aa, Homo sapiens
LRFI

SEQ ID NO: 176 - protein, 3 aa, Homo sapiens
LRF

SEQ ID NO: 177 - protein, 4 aa, Homo sapiens
RFIP

SEQ ID NO: 178 - protein, 3 aa, Homo sapiens
RFI

SEQ ID NO: 179 - protein, 3 aa, Homo sapiens
FIP

SEQ ID NO: 180 - protein, 1132 aa, Homo sapiens
MPRAPRCRAVRSLLRSHYREVLPLATFVRRLGPQGWRLVQRGDPAAFRALVAQCLVCVPWDARPPPAAPSFRQVSCLKELVARVLQRLCERGAKNVLAFGFALLDGARGGPPEAFTTSVRSYLPNTVTDALRGSGAWGLLLRRVGDDVLVHLLARCALFVLVAPSCAYQVCGPPLYQLGAATQARPPPHASGPRRRLGCERAWNHSVREAGVPLGLPAPGARRRGGSASRSLPLPKRPRRGAAPEPERTPVGQGSWAHPGRTRGPSDRGFCVVSPARPAEEATSLEGALSGTRHSHPSVGRQHHAGPPSTSRPPRPWDTPCPPVYAETKHFLYSSGDKEQLRPSFLLSSLRPSLTGARRLVETIFLGSRPWMPGTPRRLPRLPQRYWQMRPLFLELLGNHAQCPYGVLLKTHCPLRAAVTPAAGVCAREKPQGSVAAPEEEDTDPRRLVQLLRQHSSPWQVYGFVRACLRRLVPPGLWGSRHNERRFLRNTKKFISLGKHAKLSLQELTWKMSVRDCAWLRRSPGVGCVPAAEHRLREEILAKFLHWLMSVYVVELLRSFFYVTETTFQKNRLFFYRKSVWSKLQSIGIRQHLKRVQLRELSEAEVRQHREARPALLTSRLRFIPKPDGLRPIVNMDYVVGARTFRREKRAERLTSRVKALFSVLNYERARRPGLLGASVLGLDDIHRAWRTFVLRVRAQDPPPELYFVKVDVTGAYDTIPQDRLTEVIASIIKPQNTYCVRRYAVVQKAAHGHVRKAFKSHVSTLTDLQPYMRQFVAHLQETSPLRDAVVIEQSSSLNEASSGLFDVFLRFMCHHAVRIRGKSYVQCQGIPQGSILSTLLCSLCYGDMENKLFAGIRRDGLLLRLVDDFLLVTPHLTHAKTFLRTLVRGVPEYGCVVNLRKTVVNFPVEDEALGGTAFVQMPAHGLFPWCGLLLDTRTLEVQSDYSSYARTSIRASLTFNRGFKAGRNMRRKLFGVLRLKCHSLFLDLQVNSLQTVCTNIYKILLLQAYRFHACVLQLPFHQQVWKNPTFFLRVISDTASLCYSILKAKNAGMSLGAKGAAGPLPSEAVQWLCHQAFLLKLTRHRVTYVPLLGSLRTAQTQLSRKLPGTTLTALEAAANPALPSDFKTILD